European Patent Application EP 4 421 166 A1, published August 28, 2024. Title: Improved Split HaloTags. Applicant: Max-Planck-Gesellschaft. The sequence listing filed with the application follows.

SEQUENCE LISTING (377 sequences)

SEQ ID NO: 1 - protein, 305 aa, synthetic construct
FARETFQAFRTTDVGRKLIIDQNVFIEGTLPMGVVRPLTEVEMDHYREPFLNPVDREPLWRFPNELPIAGEPANIVALVEEYMDWLHQSPVPKLLFWGTPGVLIPPAEAARLAKSLPNCKAVDIGPGLNLLQEDNPDLIGSEIARWLSTLEIGGTGGSGGTGGSGGSIGTGFPFDPHYVEVLGERMHYVDVGPRDGTPVLFLHGNPTSSYVWRNIIPHVAPTHRCIAPDLIGMGKSDKPDLGYFFDDHVRFMDAFIEALGLEEVVLVIHDWGSALGFHWAKRNPERVKGIAFMEFIRPIPTWDEW

SEQ ID NO: 2 - protein, 140 aa, synthetic construct
DVGRKLIIDQNVFIEGTLPMGVVRPLTEVEMDHYREPFLNPVDREPLWRFPNELPIAGEPANIVALVEEYMDWLHQSPVPKLLFWGTPGVLIPPAEAARLAKSLPNCKAVDIGPGLNLLQEDNPDLIGSEIARWLSTLEI

SEQ ID NO: 3 - protein, 138 aa, synthetic construct
IGTGFPFDPHYVEVLGERMHYVDVGPRDGTPVLFLHGNPTSSYVWRNIIPHVAPTHRCIAPDLIGMGKSDKPDLGYFFDDHVRFMDAFIEALGLEEVVLVIHDWGSALGFHWAKRNPERVKGIAFMEFIRPIPTWDEW

SEQ ID NO: 4 - protein, 9 aa, synthetic construct
ARETFQAFR

SEQ ID NO: 5 - protein, 10 aa, synthetic construct
ARETFQAFRT

SEQ ID NO: 6 - protein, 14 aa, synthetic construct
SKRDAREMFQAFRT

SEQ ID NO: 7 - protein, 10 aa, synthetic construct
ARLFFQLFRT

SEQ ID NO: 8 - protein, 14 aa, synthetic construct
YFQGARETFQAFRT

SEQ ID NO: 9 - protein, 10 aa, synthetic construct
WIETFKLYRE

SEQ ID NO: 10 - protein, 14 aa, synthetic construct
RKKEARETFQAFRT

SEQ ID NO: 11 - protein, 10 aa, synthetic construct
VIETFKLFRS

SEQ ID NO: 12 - protein, 10 aa, synthetic construct
AREMFQLFRT

SEQ ID NO: 13 - protein, 10 aa, synthetic construct
AYKIFQLFRT

SEQ ID NO: 14 - protein, 10 aa, synthetic construct
AIRMFQLFRT

SEQ ID NO: 15 - protein, 14 aa, synthetic construct
WGDEARETFQAFRT

SEQ ID NO: 16 - protein, 10 aa, synthetic construct
AREMFQAFRT

SEQ ID NO: 17 - protein, 14 aa, synthetic construct
WKDEVIDAFRKFRE

SEQ ID NO: 18 - protein, 10 aa, synthetic construct
ERETWQAFRT

SEQ ID NO: 19 - protein, 14 aa, synthetic construct
WREEVRKTFKLFRQ

SEQ ID NO: 20 - protein, 10 aa, synthetic construct
WREMFRLFRT

SEQ ID NO: 21 - protein, 14 aa, synthetic construct
YFQGAREMFQAFRT

SEQ ID NO: 22 - protein, 14 aa, synthetic construct
WKEEVIKAFKLFRD

SEQ ID NO: 23 - protein, 10 aa, synthetic construct
AVNMFQLFRT

SEQ ID NO: 24 - protein, 14 aa, synthetic construct
WREEVRKAFKLFRS

SEQ ID NO: 25 - protein, 14 aa, synthetic construct
WREEVRKAFKLFRQ

SEQ ID NO: 26 - protein, 10 aa, synthetic construct
WRETFQLFRT

SEQ ID NO: 27 - protein, 14 aa, synthetic construct
WREMFRLFRTGRVQ

SEQ ID NO: 28 - protein, 10 aa, synthetic construct
WREMFQAFRT

SEQ ID NO: 29 - protein, 14 aa, synthetic construct
WREMFRLFRTGQRS

SEQ ID NO: 30 - protein, 10 aa, synthetic construct
WREMFQLFRT

SEQ ID NO: 31 - protein, 14 aa, synthetic construct
SKRDWREMFRLFRT

SEQ ID NO: 32 - protein, 14 aa, synthetic construct
RVMSWREMFRLFRT

SEQ ID NO: 33 - protein, 14 aa, synthetic construct
RMWSWREMFRLFRT

SEQ ID NO: 34 - protein, 14 aa, synthetic construct
WKRDWREMFRLFRT

SEQ ID NO: 35 - protein, 14 aa, synthetic construct
RQWTWREMFRLFRT

SEQ ID NO: 36 - protein, 14 aa, synthetic construct
RGWTWREMFRLFRT

SEQ ID NO: 37 - protein, 14 aa, synthetic construct
RMWTWREMFRLFRT

SEQ ID NO: 38 - protein, 14 aa, synthetic construct
RQWSWREMFRLFRT

SEQ ID NO: 39 - protein, 14 aa, synthetic construct
RGWSWREMFRLFRT

SEQ ID NO: 40 - protein, 14 aa, synthetic construct
WKRDARETFQAFRT

SEQ ID NO: 41 - protein, 14 aa, synthetic construct
WREEVRKAFKLFRD

SEQ ID NO: 42 - protein, 10 aa, synthetic construct
AIRMFQLFRE

SEQ ID NO: 43 - protein, 14 aa, synthetic construct
LSEEARETFQAFRT

SEQ ID NO: 44 - protein, 14 aa, synthetic construct
WKREARETFQAFRT

SEQ ID NO: 45 - protein, 14 aa, synthetic construct
WSKEARETFQAFRT

SEQ ID NO: 46 - protein, 14 aa, synthetic construct
WDKEARETFQAFRT

SEQ ID NO: 47 - protein, 14 aa, synthetic construct
WREEVRKTFKLFRS

SEQ ID NO: 48 - protein, 14 aa, synthetic construct
SKRDARETFQAFRT

SEQ ID NO: 49 - protein, 14 aa, synthetic construct
WKEKARETFQAFRT

SEQ ID NO: 50 - protein, 10 aa, synthetic construct
VREAFKLFRS

SEQ ID NO: 51 - protein, 10 aa, synthetic construct
AREAFKAFRS

SEQ ID NO: 52 - protein, 14 aa, synthetic construct
DKETARETFQAFRT

SEQ ID NO: 53 - protein, 14 aa, synthetic construct
DGEDARETFQAFRT

SEQ ID NO: 54 - protein, 14 aa, synthetic construct
QERDARETFQAFRT

SEQ ID NO: 55 - protein, 10 aa, synthetic construct
LRKTFKLFRS

SEQ ID NO: 56 - protein, 14 aa, synthetic construct
WRETARETFQAFRT

SEQ ID NO: 57 - protein, 10 aa, synthetic construct
LIETFKLFRS

SEQ ID NO: 58 - protein, 14 aa, synthetic construct
WEETARETFQAFRT

SEQ ID NO: 59 - protein, 10 aa, synthetic construct
LIKTFQLFRQ

SEQ ID NO: 60 - protein, 14 aa, synthetic construct
WKETARETFQAFRT

SEQ ID NO: 61 - protein, 10 aa, synthetic construct
AQEAFKAFRS

SEQ ID NO: 62 - protein, 10 aa, synthetic construct
IRDAFQAFRS

SEQ ID NO: 63 - protein, 10 aa, synthetic construct
AIKAFQLFRS

SEQ ID NO: 64 - protein, 14 aa, synthetic construct
WDREARETFQAFRT

SEQ ID NO: 65 - protein, 14 aa, synthetic construct
FKQDARETFQAFRT

SEQ ID NO: 66 - protein, 10 aa, synthetic construct
ARDMFIKFRD

SEQ ID NO: 67 - protein, 14 aa, synthetic construct
WRKEARETFQAFRT

SEQ ID NO: 68 - protein, 14 aa, synthetic construct
YKDDLIKTFILFRQ

SEQ ID NO: 69 - protein, 14 aa, synthetic construct
LGEEARETFQAFRT

SEQ ID NO: 70 - protein, 14 aa, synthetic construct
YKEDLIKTFILFRQ

SEQ ID NO: 71 - protein, 14 aa, synthetic construct
WKEEVIKAFKLFRS

SEQ ID NO: 72 - protein, 10 aa, synthetic construct
SRDTFQAFRS

SEQ ID NO: 73 - protein, 14 aa, synthetic construct
WKKEARETFQAFRT

SEQ ID NO: 74 - protein, 14 aa, synthetic construct
DGRDARETFQAFRT

SEQ ID NO: 75 - protein, 10 aa, synthetic construct
WRETFQAFRT

SEQ ID NO: 76 - protein, 14 aa, synthetic construct
WKEEVIKAFKLFRQ

SEQ ID NO: 77 - protein, 10 aa, synthetic construct
LIKAFQLFRS

SEQ ID NO: 78 - protein, 14 aa, synthetic construct
SKKEARETFQAFRT

SEQ ID NO: 79 - protein, 14 aa, synthetic construct
WREEVIKAFKLFRQ

SEQ ID NO: 80 - protein, 14 aa, synthetic construct
WDEEVKDAFKKFRD

SEQ ID NO: 81 - protein, 14 aa, synthetic construct
WKEEVIKAFRLFRE

SEQ ID NO: 82 - protein, 10 aa, synthetic construct
LIKTFQLFRS

SEQ ID NO: 83 - protein, 10 aa, synthetic construct
ARKAFELFRS

SEQ ID NO: 84 - protein, 10 aa, synthetic construct
SRDAFKAFRS

SEQ ID NO: 85 - protein, 10 aa, synthetic construct
LIKTFQLYRS

SEQ ID NO: 86 - protein, 14 aa, synthetic construct
YSEEARETFQAFRT

SEQ ID NO: 87 - protein, 14 aa, synthetic construct
RDEDARETFQAFRT

SEQ ID NO: 88 - protein, 10 aa, synthetic construct
VRTAFKLFRS

SEQ ID NO: 89 - protein, 10 aa, synthetic construct
SRDAFKAYRS

SEQ ID NO: 90 - protein, 10 aa, synthetic construct
TRDTFQAFQS

SEQ ID NO: 91 - protein, 14 aa, synthetic construct
WEKEARETFQAFRT

SEQ ID NO: 92 - protein, 14 aa, synthetic construct
WKEEVIKAFRLYRE

SEQ ID NO: 93 - protein, 10 aa, synthetic construct
LVETFKLFRS

SEQ ID NO: 94 - protein, 14 aa, synthetic construct
WKEDVIDAFRKFRD

SEQ ID NO: 95 - protein, 14 aa, synthetic construct
LGDDARETFQAFRT

SEQ ID NO: 96 - protein, 14 aa, synthetic construct
MKEDARETFQAFRT

SEQ ID NO: 97 - protein, 10 aa, synthetic construct
VVKTFQLFRS

SEQ ID NO: 98 - protein, 10 aa, synthetic construct
ARETFQAFRS

SEQ ID NO: 99 - protein, 14 aa, synthetic construct
FGKEARETFQAFRT

SEQ ID NO: 100 - protein, 14 aa, synthetic construct
WKELARETFQAFRT

SEQ ID NO: 101 - protein, 14 aa, synthetic construct
WKEEVIKAFIKFRE

SEQ ID NO: 102 - protein, 10 aa, synthetic construct
VREAFKLFRQ

SEQ ID NO: 103 - protein, 10 aa, synthetic construct
SREAFEAFRS

SEQ ID NO: 104 - protein, 14 aa, synthetic construct
WKEDARETFQAFRT

SEQ ID NO: 105 - protein, 10 aa, synthetic construct
VIKTFQLFRS

SEQ ID NO: 106 - protein, 14 aa, synthetic construct
LAEDARETFQAFRT

SEQ ID NO: 107 - protein, 10 aa, synthetic construct
LIETFRLFRQ

SEQ ID NO: 108 - protein, 14 aa, synthetic construct
HKEEARETFQAFRT

SEQ ID NO: 109 - protein, 14 aa, synthetic construct
WGRDARETFQAFRT

SEQ ID NO: 110 - protein, 10 aa, synthetic construct
GRETFQAFRS

SEQ ID NO: 111 - protein, 10 aa, synthetic construct
ARETFQKFRT

SEQ ID NO: 112 - protein, 10 aa, synthetic construct
IRETFQAFRT

SEQ ID NO: 113 - protein, 14 aa, synthetic construct
QKKEARETFQAFRT

SEQ ID NO: 114 - protein, 14 aa, synthetic construct
WKEEVIKAFILYRS

SEQ ID NO: 115 - protein, 14 aa, synthetic construct
WYEEARETFQAFRT

SEQ ID NO: 116 - protein, 10 aa, synthetic construct
VIKAFQLFRQ

SEQ ID NO: 117 - protein, 14 aa, synthetic construct
FGREARETFQAFRT

SEQ ID NO: 118 - protein, 14 aa, synthetic construct
WKEEVIKAFRLYRD

SEQ ID NO: 119 - protein, 10 aa, synthetic construct
TRDTFQAFRS

SEQ ID NO: 120 - protein, 14 aa, synthetic construct
YKDDARETFQAFRT

SEQ ID NO: 121 - protein, 10 aa, synthetic construct
AIKTFQLFRS

SEQ ID NO: 122 - protein, 10 aa, synthetic construct
ARETFQAYRS

SEQ ID NO: 123 - protein, 10 aa, synthetic construct
SRDTFRAFRS

SEQ ID NO: 124 - protein, 14 aa, synthetic construct
HKDEARETFQAFRT

SEQ ID NO: 125 - protein, 10 aa, synthetic construct
TRETFKAFRS

SEQ ID NO: 126 - protein, 10 aa, synthetic construct
SRDTFQAFRT

SEQ ID NO: 127 - protein, 10 aa, synthetic construct
VIKTFQLFRQ

SEQ ID NO: 128 - protein, 10 aa, synthetic construct
SRDAFQAFRS

SEQ ID NO: 129 - protein, 14 aa, synthetic construct
WKEEVIKAFILYRQ

SEQ ID NO: 130 - protein, 14 aa, synthetic construct
QREEARETFQAFRT

SEQ ID NO: 131 - protein, 10 aa, synthetic construct
AQETFKAYRS

SEQ ID NO: 132 - protein, 14 aa, synthetic construct
WDRDARETFQAFRT

SEQ ID NO: 133 - protein, 10 aa, synthetic construct
ARDTFRAFRS

SEQ ID NO: 134 - protein, 14 aa, synthetic construct
MKEEARETFQAFRT

SEQ ID NO: 135 - protein, 14 aa, synthetic construct
WHEEARETFQAFRT

SEQ ID NO: 136 - protein, 10 aa, synthetic construct
AVETFKLFRQ

SEQ ID NO: 137 - protein, 14 aa, synthetic construct
DKEDARETFQAFRT

SEQ ID NO: 138 - protein, 10 aa, synthetic construct
FIETFKLFRD

SEQ ID NO: 139 - protein, 14 aa, synthetic construct
WDEDARETFQAFRT

SEQ ID NO: 140 - protein, 14 aa, synthetic construct
LKEEARETFQAFRT

SEQ ID NO: 141 - protein, 10 aa, synthetic construct
ARDTFQAFRS

SEQ ID NO: 142 - protein, 14 aa, synthetic construct
WAQEARETFQAFRT

SEQ ID NO: 143 - protein, 14 aa, synthetic construct
SGEDARETFQAFRT

SEQ ID NO: 144 - protein, 10 aa, synthetic construct
TREAFKAFRA

SEQ ID NO: 145 - protein, 14 aa, synthetic construct
LKEDARETFQAFRT

SEQ ID NO: 146 - protein, 14 aa, synthetic construct
LGEDARETFQAFRT

SEQ ID NO: 147 - protein, 14 aa, synthetic construct
YGEELIKMFIKFRD

SEQ ID NO: 148 - protein, 14 aa, synthetic construct
WSEEARETFQAFRT

SEQ ID NO: 149 - protein, 14 aa, synthetic construct
MSEEARETFQAFRT

SEQ ID NO: 150 - protein, 14 aa, synthetic construct
FSEDARETFQAFRT

SEQ ID NO: 151 - protein, 14 aa, synthetic construct
SKEIARETFQAFRT

SEQ ID NO: 152 - protein, 10 aa, synthetic construct
AIRTFQLFRQ

SEQ ID NO: 153 - protein, 14 aa, synthetic construct
WEEEARETFQAFRT

SEQ ID NO: 154 - protein, 14 aa, synthetic construct
SRDEARETFQAFRT

SEQ ID NO: 155 - protein, 10 aa, synthetic construct
TRDTFQAFRT

SEQ ID NO: 156 - protein, 10 aa, synthetic construct
SRETFQAFRT

SEQ ID NO: 157 - protein, 14 aa, synthetic construct
MREDARETFQAFRT

SEQ ID NO: 158 - protein, 14 aa, synthetic construct
RKEEARETFQAFRT

SEQ ID NO: 159 - protein, 14 aa, synthetic construct
YKEIARETFQAFRT

SEQ ID NO: 160 - protein, 10 aa, synthetic construct
ARETFQLFRT

SEQ ID NO: 161 - protein, 14 aa, synthetic construct
KDETARETFQAFRT

SEQ ID NO: 162 - protein, 10 aa, synthetic construct
VIRMFQLFRE

SEQ ID NO: 163 - protein, 14 aa, synthetic construct
FKEDARETFQAFRT

SEQ ID NO: 164 - protein, 14 aa, synthetic construct
LKDIARETFQAFRT

SEQ ID NO: 165 - protein, 14 aa, synthetic construct
WGEIARETFQAFRT

SEQ ID NO: 166 - protein, 14 aa, synthetic construct
WGEEARETFQAFRT

SEQ ID NO: 167 - protein, 10 aa, synthetic construct
ARRTFQAFRT

SEQ ID NO: 168 - protein, 14 aa, synthetic construct
WGEDARETFQAFRT

SEQ ID NO: 169 - protein, 14 aa, synthetic construct
KKEEARETFQAFRT

SEQ ID NO: 170 - protein, 14 aa, synthetic construct
YGEDARETFQAFRT

SEQ ID NO: 171 - protein, 10 aa, synthetic construct
IRDTFQAYRS

SEQ ID NO: 172 - protein, 14 aa, synthetic construct
YWEEARETFQAFRT

SEQ ID NO: 173 - protein, 10 aa, synthetic construct
AREFFQAFRT

SEQ ID NO: 174 - protein, 14 aa, synthetic construct
WKEIARETFQAFRT

SEQ ID NO: 175 - protein, 10 aa, synthetic construct
VRETFQAFRT

SEQ ID NO: 176 - protein, 14 aa, synthetic construct
WDEEARETFQAFRT

SEQ ID NO: 177 - protein, 10 aa, synthetic construct
LIDTFRKFRS

SEQ ID NO: 178 - protein, 14 aa, synthetic construct
WSEDARETFQAFRT

SEQ ID NO: 179 - protein, 14 aa, synthetic construct
FSEEARETFQAFRT

SEQ ID NO: 180 - protein, 14 aa, synthetic construct
QKDVARETFQAFRT

SEQ ID NO: 181 - protein, 14 aa, synthetic construct
WNEEARETFQAFRT

SEQ ID NO: 182 - protein, 10 aa, synthetic construct
ARETFQAYRT

SEQ ID NO: 183 - protein, 14 aa, synthetic construct
FAEDARETFQAFRT

SEQ ID NO: 184 - protein, 10 aa, synthetic construct
ARETFKAFRS

SEQ ID NO: 185 - protein, 14 aa, synthetic construct
EKEDARETFQAFRT

SEQ ID NO: 186 - protein, 10 aa, synthetic construct
LIEAFKLFRD

SEQ ID NO: 187 - protein, 14 aa, synthetic construct
STEEARETFQAFRT

SEQ ID NO: 188 - protein, 14 aa, synthetic construct
WTEEARETFQAFRT

SEQ ID NO: 189 - protein, 10 aa, synthetic construct
LRETFQAFRT

SEQ ID NO: 190 - protein, 14 aa, synthetic construct
FTEEARETFQAFRT

SEQ ID NO: 191 - protein, 14 aa, synthetic construct
WDEIARETFQAFRT

SEQ ID NO: 192 - protein, 14 aa, synthetic construct
FGEEARETFQAFRT

SEQ ID NO: 193 - protein, 14 aa, synthetic construct
WLEEARETFQAFRT

SEQ ID NO: 194 - protein, 14 aa, synthetic construct
DAEDARETFQAFRT

SEQ ID NO: 195 - protein, 10 aa, synthetic construct
ARETFRAFRT

SEQ ID NO: 196 - protein, 14 aa, synthetic construct
FREEARETFQAFRT

SEQ ID NO: 197 - protein, 10 aa, synthetic construct
LIETFKLFRE

SEQ ID NO: 198 - protein, 14 aa, synthetic construct
WKDDARETFQAFRT

SEQ ID NO: 199 - protein, 14 aa, synthetic construct
YREEARETFQAFRT

SEQ ID NO: 200 - protein, 10 aa, synthetic construct
VIKAFQLFRE

SEQ ID NO: 201 - protein, 14 aa, synthetic construct
DGEIARETFQAFRT

SEQ ID NO: 202 - protein, 14 aa, synthetic construct
YGEEARETFQAFRT

SEQ ID NO: 203 - protein, 14 aa, synthetic construct
ESEDARETFQAFRT

SEQ ID NO: 204 - protein, 14 aa, synthetic construct
PKEDARETFQAFRT

SEQ ID NO: 205 - protein, 14 aa, synthetic construct
FGDEARETFQAFRT

SEQ ID NO: 206 - protein, 14 aa, synthetic construct
QGEEARETFQAFRT

SEQ ID NO: 207 - protein, 14 aa, synthetic construct
TGEDARETFQAFRT

SEQ ID NO: 208 - protein, 14 aa, synthetic construct
QAEEARETFQAFRT

SEQ ID NO: 209 - protein, 14 aa, synthetic construct
FQEEARETFQAFRT

SEQ ID NO: 210 - protein, 10 aa, synthetic construct
TREAFEAFRS

SEQ ID NO: 211 - protein, 14 aa, synthetic construct
WKEEVVKAFIKFRD

SEQ ID NO: 212 - protein, 14 aa, synthetic construct
WFDEARETFQAFRT

SEQ ID NO: 213 - protein, 14 aa, synthetic construct
DGEEARETFQAFRT

SEQ ID NO: 214 - protein, 10 aa, synthetic construct
AKETFQAFRT

SEQ ID NO: 215 - protein, 14 aa, synthetic construct
ARETFQAFRTALKD

SEQ ID NO: 216 - protein, 14 aa, synthetic construct
WEDEARETFQAFRT

SEQ ID NO: 217 - protein, 14 aa, synthetic construct
DKEEARETFQAFRT

SEQ ID NO: 218 - protein, 14 aa, synthetic construct
DGDDARETFQAFRT

SEQ ID NO: 219 - protein, 14 aa, synthetic construct
FKEEARETFQAFRT

SEQ ID NO: 220 - protein, 10 aa, synthetic construct
VIETFKLFRD

SEQ ID NO: 221 - protein, 10 aa, synthetic construct
LIETFIQYRQ

SEQ ID NO: 222 - protein, 10 aa, synthetic construct
GRETFQAFRT

SEQ ID NO: 223 - protein, 14 aa, synthetic construct
WADEARETFQAFRT

SEQ ID NO: 224 - protein, 10 aa, synthetic construct
ARETFKAFRD

SEQ ID NO: 225 - protein, 14 aa, synthetic construct
WTDEARETFQAFRT

SEQ ID NO: 226 - protein, 10 aa, synthetic construct
SRETFEAFRS

SEQ ID NO: 227 - protein, 14 aa, synthetic construct
YQEEARETFQAFRT

SEQ ID NO: 228 - protein, 10 aa, synthetic construct
TRETFQAFRT

SEQ ID NO: 229 - protein, 10 aa, synthetic construct
AIEAFKLFRE

SEQ ID NO: 230 - protein, 10 aa, synthetic construct
ARDTFQAFRT

SEQ ID NO: 231 - protein, 14 aa, synthetic construct
YKEDARETFQAFRT

SEQ ID NO: 232 - protein, 14 aa, synthetic construct
WREIARETFQAFRT

SEQ ID NO: 233 - protein, 14 aa, synthetic construct
YGEIARETFQAFRT

SEQ ID NO: 234 - protein, 14 aa, synthetic construct
FKEIARETFQAFRT

SEQ ID NO: 235 - protein, 14 aa, synthetic construct
FSDEARETFQAFRT

SEQ ID NO: 236 - protein, 10 aa, synthetic construct
VRDTFQAFRT

SEQ ID NO: 237 - protein, 14 aa, synthetic construct
MGEDARETFQAFRT

SEQ ID NO: 238 - protein, 14 aa, synthetic construct
YKEEARETFQAFRT

SEQ ID NO: 239 - protein, 10 aa, synthetic construct
LIETFKKFRD

SEQ ID NO: 240 - protein, 10 aa, synthetic construct
GRDTFKAFRS

SEQ ID NO: 241 - protein, 14 aa, synthetic construct
WKEEVIKAFILYRE

SEQ ID NO: 242 - protein, 14 aa, synthetic construct
YAEIARETFQAFRT

SEQ ID NO: 243 - protein, 14 aa, synthetic construct
YEEEARETFQAFRT

SEQ ID NO: 244 - protein, 10 aa, synthetic construct
SRETFILFRQ

SEQ ID NO: 245 - protein, 10 aa, synthetic construct
AQETFKAFRD

SEQ ID NO: 246 - protein, 10 aa, synthetic construct
ARETFQAFRQ

SEQ ID NO: 247 - protein, 10 aa, synthetic construct
LIKTFQLFRD

SEQ ID NO: 248 - protein, 14 aa, synthetic construct
DKEIARETFQAFRT

SEQ ID NO: 249 - protein, 10 aa, synthetic construct
LIETFRQFRE

SEQ ID NO: 250 - protein, 10 aa, synthetic construct
ARDTFRAFRD

SEQ ID NO: 251 - protein, 14 aa, synthetic construct
WSEMARETFQAFRT

SEQ ID NO: 252 - protein, 14 aa, synthetic construct
ARETFQAFRTIFEH

SEQ ID NO: 253 - protein, 10 aa, synthetic construct
ARETFKAFRT

SEQ ID NO: 254 - protein, 14 aa, synthetic construct
WREEARETFQAFRT

SEQ ID NO: 255 - protein, 10 aa, synthetic construct
ARETFIAFRT

SEQ ID NO: 256 - protein, 14 aa, synthetic construct
WKDEARETFQAFRT

SEQ ID NO: 257 - protein, 14 aa, synthetic construct
WGQEARETFQAFRT

SEQ ID NO: 258 - protein, 14 aa, synthetic construct
WSDEARETFQAFRT

SEQ ID NO: 259 - protein, 14 aa, synthetic construct
WRDEARETFQAFRT

SEQ ID NO: 260 - protein, 10 aa, synthetic construct
ARETFQAFRD

SEQ ID NO: 261 - protein, 10 aa, synthetic construct
LIETFKLFRQ

SEQ ID NO: 262 - protein, 14 aa, synthetic construct
SSEEARETFQAFRT

SEQ ID NO: 263 - protein, 14 aa, synthetic construct
WSETARETFQAFRT

SEQ ID NO: 264 - protein, 14 aa, synthetic construct
FKDDARETFQAFRT

SEQ ID NO: 265 - protein, 14 aa, synthetic construct
NGEDARETFQAFRT

SEQ ID NO: 266 - protein, 10 aa, synthetic construct
TRETFEAFRS

SEQ ID NO: 267 - protein, 14 aa, synthetic construct
WQEEARETFQAFRT

SEQ ID NO: 268 - protein, 14 aa, synthetic construct
SKEEARETFQAFRT

SEQ ID NO: 269 - protein, 10 aa, synthetic construct
AREAFEAFRS

SEQ ID NO: 270 - protein, 10 aa, synthetic construct
AIKAFQLFRE

SEQ ID NO: 271 - protein, 10 aa, synthetic construct
TRETFEAFQS

SEQ ID NO: 272 - protein, 14 aa, synthetic construct
KEEEARETFQAFRT

SEQ ID NO: 273 - protein, 14 aa, synthetic construct
YNEEARETFQAFRT

SEQ ID NO: 274 - protein, 10 aa, synthetic construct
SRDTFKAFQT

SEQ ID NO: 275 - protein, 14 aa, synthetic construct
WWEEARETFQAFRT

SEQ ID NO: 276 - protein, 10 aa, synthetic construct
AVEMFKLFRD

SEQ ID NO: 277 - protein, 10 aa, synthetic construct
MRETFQAFRT

SEQ ID NO: 278 - protein, 10 aa, synthetic construct
VRKTFELFRS

SEQ ID NO: 279 - protein, 10 aa, synthetic construct
SRDTFKAFQS

SEQ ID NO: 280 - protein, 14 aa, synthetic construct
YTEEARETFQAFRT

SEQ ID NO: 281 - protein, 10 aa, synthetic construct
AIEAFKLFRQ

SEQ ID NO: 282 - protein, 14 aa, synthetic construct
QKDEARETFQAFRT

SEQ ID NO: 283 - protein, 14 aa, synthetic construct
KSEEARETFQAFRT

SEQ ID NO: 284 - protein, 10 aa, synthetic construct
AIETFKLFRQ

SEQ ID NO: 285 - protein, 14 aa, synthetic construct
WAEEARETFQAFRT

SEQ ID NO: 286 - protein, 14 aa, synthetic construct
WTKEARETFQAFRT

SEQ ID NO: 287 - protein, 10 aa, synthetic construct
VRDTFQAFRS

SEQ ID NO: 288 - protein, 10 aa, synthetic construct
VRKTFKLFRQ

SEQ ID NO: 289 - protein, 14 aa, synthetic construct
MGEEARETFQAFRT

SEQ ID NO: 290 - protein, 14 aa, synthetic construct
STEIARETFQAFRT

SEQ ID NO: 291 - protein, 10 aa, synthetic construct
SRDTFQAFQS

SEQ ID NO: 292 - protein, 10 aa, synthetic construct
VIRTFQLFRQ

SEQ ID NO: 293 - protein, 10 aa, synthetic construct
SRDAFQAYRS

SEQ ID NO: 294 - protein, 10 aa, synthetic construct
LIETFKLFRT

SEQ ID NO: 295 - protein, 10 aa, synthetic construct
VREFFKLARD

SEQ ID NO: 296 - protein, 14 aa, synthetic construct
WAKEARETFQAFRT

SEQ ID NO: 297 - protein, 10 aa, synthetic construct
NRDTFQAFRS

SEQ ID NO: 298 - protein, 10 aa, synthetic construct
VRETFKLFRS

SEQ ID NO: 299 - protein, 10 aa, synthetic construct
IRETFEAFRS

SEQ ID NO: 300 - protein, 14 aa, synthetic construct
YKEELIKTFRLFMQ

SEQ ID NO: 301 - protein, 10 aa, synthetic construct
AIKTFILFRE

SEQ ID NO: 302 - protein, 10 aa, synthetic construct
AREAFQAFRT

SEQ ID NO: 303 - protein, 14 aa, synthetic construct
KDEEARETFQAFRT

SEQ ID NO: 304 - protein, 10 aa, synthetic construct
LIEAFRQFRS

SEQ ID NO: 305 - protein, 10 aa, synthetic construct
VIRAFQLFRQ

SEQ ID NO: 306 - protein, 14 aa, synthetic construct
WGKEARETFQAFRT

SEQ ID NO: 307 - protein, 10 aa, synthetic construct
VRTAFKLFRQ

SEQ ID NO: 308 - protein, 10 aa, synthetic construct
SRDTFKAFRS

SEQ ID NO: 309 - protein, 10 aa, synthetic construct
AIETFKLFRE

SEQ ID NO: 310 - protein, 10 aa, synthetic construct
VVETFKLFRS

SEQ ID NO: 311 - protein, 10 aa, synthetic construct
ARDTFILFRE

SEQ ID NO: 312 - protein, 10 aa, synthetic construct
VRDTFILFRS

SEQ ID NO: 313 - protein, 14 aa, synthetic construct
YKEDLIDTFRKFRQ

SEQ ID NO: 314 - protein, 10 aa, synthetic construct
VIKAFQLFRS

SEQ ID NO: 315 - protein, 14 aa, synthetic construct
ARETFQAFRTAHQK

SEQ ID NO: 316 - protein, 14 aa, synthetic construct
SSEDARETFQAFRT

SEQ ID NO: 317 - protein, 10 aa, synthetic construct
IREAFEAFRS

SEQ ID NO: 318 - protein, 10 aa, synthetic construct
IREAFEAYRS

SEQ ID NO: 319 - protein, 14 aa, synthetic construct
SKEDARETFQAFRT

SEQ ID NO: 320 - protein, 10 aa, synthetic construct
ARDTFKAFRS

SEQ ID NO: 321 - protein, 10 aa, synthetic construct
AQETFKAFRS

SEQ ID NO: 322 - protein, 14 aa, synthetic construct
FWEEARETFQAFRT

SEQ ID NO: 323 - protein, 10 aa, synthetic construct
VVRTFKLFRS

SEQ ID NO: 324 - protein, 14 aa, synthetic construct
LAEEARETFQAFRT

SEQ ID NO: 325 - protein, 10 aa, synthetic construct
VIKAFIKFRE

SEQ ID NO: 326 - protein, 14 aa, synthetic construct
EKEEARETFQAFRT

SEQ ID NO: 327 - protein, 10 aa, synthetic construct
GRDTFQAFRS

SEQ ID NO: 328 - protein, 14 aa, synthetic construct
KKEDARETFQAFRT

SEQ ID NO: 329 - protein, 14 aa, synthetic construct
ARETFQAFRTGASS

SEQ ID NO: 330 - protein, 10 aa, synthetic construct
LIKTFILFRD

SEQ ID NO: 331 - protein, 10 aa, synthetic construct
ARKTFQAFRT

SEQ ID NO: 332 - protein, 14 aa, synthetic construct
QKEDARETFQAFRT

SEQ ID NO: 333 - protein, 14 aa, synthetic construct
MRDEARETFQAFRT

SEQ ID NO: 334 - protein, 10 aa, synthetic construct
GRDTFKAFQS

SEQ ID NO: 335 - protein, 10 aa, synthetic construct
AIRAFQLFRQ

SEQ ID NO: 336 - protein, 14 aa, synthetic construct
YGRDARETFQAFRT

SEQ ID NO: 337 - protein, 14 aa, synthetic construct
RGWSAREMFQAFRT

SEQ ID NO: 338 - protein, 14 aa, synthetic construct
RGWSARETFQAFRT

SEQ ID NO: 339 - protein, 14 aa, synthetic construct
RMWTAREMFQAFRT

SEQ ID NO: 340 - protein, 14 aa, synthetic construct
RQWSARETFQAFRT

SEQ ID NO: 341 - protein, 14 aa, synthetic construct
WKRDAREMFQAFRT

SEQ ID NO: 342 - protein, 14 aa, synthetic construct
LSEEAREMFQAFRT

SEQ ID NO: 343 - protein, 14 aa, synthetic construct
RQWSAREMFQAFRT

SEQ ID NO: 344 - protein, 22 aa, synthetic construct
RSDDPRKTQTIASKISRDLNGS

SEQ ID NO: 345 - protein, 22 aa, synthetic construct
KGGTKRDADKAVRDTLLSLNGQ

SEQ ID NO: 346 - protein, 22 aa, synthetic construct
GGAPRDEALKKIEKAKRDTGDQ

SEQ ID NO: 347 - protein, 23 aa, synthetic construct
KSKYDRDQILKIIAELEKKTGGS

SEQ ID NO: 348 - protein, 23 aa, synthetic construct
QSKYPPEWLEKVIRELLKRKNGR

SEQ ID NO: 349 - protein, 23 aa, synthetic construct
KSKYDKRQIRDIADKIAKDNNHQ

SEQ ID NO: 350 - protein, 22 aa, synthetic construct
GADDKTKIEKILEEIKRRWQGR

SEQ ID NO: 351 - protein, 22 aa, synthetic construct
GTSDPRNQEIAKKLARDASTVP

SEQ ID NO: 352 - protein, 22 aa, synthetic construct
NGADKEQIDRAIEKAKRDLNNQ

SEQ ID NO: 353 - protein, 23 aa, synthetic construct
KGASDRDEAKKLADDIRKKKGDQ

SEQ ID NO: 354 - protein, 23 aa, synthetic construct
NSNGHRDELEKILQTIRKQNNDI

SEQ ID NO: 355 - protein, 23 aa, synthetic construct
LKDERQRDKALEIADRADKYPTS

SEQ ID NO: 356 - protein, 23 aa, synthetic construct
KGAEDAKERLERGDIEKKKKEQP

SEQ ID NO: 357 - protein, 23 aa, synthetic construct
KGAEDAKERLERGDLDRWSQEWR

SEQ ID NO: 358 - protein, 23 aa, synthetic construct
KGAEDAKERLERRDLDKINSRNS

SEQ ID NO: 359 - protein, 23 aa, synthetic construct
KGAEDAKERLEKGYIDDKASKQQ

SEQ ID NO: 360 - protein, 23 aa, synthetic construct
KGAEDAKERLEKGELEKKWKDHP

SEQ ID NO: 361 - protein, 23 aa, synthetic construct
KGAEDAKERLERGEMEKAVKHGS

SEQ ID NO: 362 - protein, 24 aa, synthetic construct
KGAEDAKERLERDELTRDIKTYPY

SEQ ID NO: 363 - protein, 24 aa, synthetic construct
KGAEDAKERLEQGMLEEIKKKYPE

SEQ ID NO: 364 - protein, 24 aa, synthetic construct
KGAEDAKERLERDELTKIAKNLGG

SEQ ID NO: 365 - protein, 24 aa, synthetic construct
KGAEDAKERLEKNALDKIAKSKGD

SEQ ID NO: 366 - protein, 24 aa, synthetic construct
KGAEDAKERLEKNDETLKKAKDKP

SEQ ID NO: 367 - protein, 293 aa, synthetic construct
DVGRKLIIDQNVFIEGTLPMGVVRPLTEVEMDHYREPFLNPVDREPLWRFPNELPIAGEPANIVALVEEYMDWLHQSPVPKLLFWGTPGVLIPPAEAARLAKSLPNCKAVDIGPGLNLLQEDNPDLIGSEIARWLSTLEIGGTGGSGGTGGSGGSIGTGFPFDPHYVEVLGERMHYVDVGPRDGTPVLFLHGNPTSSYVWRNIIPHVAPTHRCIAPDLIGMGKSDKPDLGYFFDDHVRFMDAFIEALGLEEVVLVIHDWGSALGFHWAKRNPERVKGIAFMEFIRPIPTWDEW

SEQ ID NO: 368 - protein, 15 aa, synthetic construct
GGTGGSGGTGGSGGS

SEQ ID NO: 369 - protein, 14 aa, synthetic construct
YFQGWREMFQAFRT

SEQ ID NO: 370 - protein, 138 aa, synthetic construct
IGTGFPFDPHYVEVLGERMHYVDVGPRDGTPVLFLHGNPTSSYVWRNIIPHVAPTHRCIAPDLIGMGKSDKPDLGYFFDDHVRFMDAFIEALGLEEVVLVIHAWGSALGFHWAKRNPERVKGIAFMEFIRPIPTWDEW

SEQ ID NO: 371 - protein, 293 aa, synthetic construct
DVGRKLIIDQNVFIEGTLPMGVVRPLTEVEMDHYREPFLNPVDREPLWRFPNELPIAGEPANIVALVEEYMDWLHQSPVPKLLFWGTPGVLIPPAEAARLAKSLPNCKAVDIGPGLNLLQEDNPDLIGSEIARWLSTLEIGGTGGSGGTGGSGGSIGTGFPFDPHYVEVLGERMHYVDVGPRDGTPVLFLHGNPTSSYVWRNIIPHVAPTHRCIAPDLIGMGKSDKPDLGYFFDDHVRFMDAFIEALGLEEVVLVIHAWGSALGFHWAKRNPERVKGIAFMEFIRPIPTWDEW

SEQ ID NO: 372 - protein, 4 aa, synthetic construct
LKPG

SEQ ID NO: 373 - protein, 4 aa, synthetic construct
EKKG

SEQ ID NO: 374 - protein, 4 aa, synthetic construct
PDYE

SEQ ID NO: 375 - protein, 4 aa, synthetic construct
GDVE

SEQ ID NO: 376 - protein, 4 aa, synthetic construct
PDSN

SEQ ID NO: 377 - protein, 4 aa, synthetic construct
PDPQ